European Patent Application EP 4 782 551 A1, published July 29, 2026. Title: METHODS, KITS, AND SYSTEMS FOR IDENTIFICATION OF VECTOR COPY NUMBER AND INTEGRATION SITES. Applicant: National Resilience, Inc. Application US. The sequence listing filed with the application follows.

SEQUENCE LISTING (34 sequences)

SEQ ID NO: 1 - DNA, 36 bp, synthetic construct
  source 1..36: mol_type = other DNA
tcgtcggcagcgtcgcagctgtagatcttagccact

SEQ ID NO: 2 - DNA, 35 bp, synthetic construct
  source 1..35: mol_type = other DNA
tcgtcggcagcgtcgggactggaagggctaattca

SEQ ID NO: 3 - DNA, 36 bp, synthetic construct
  source 1..36: mol_type = other DNA
tcgtcggcagcgtcccaacgaagacaagatctgctt

SEQ ID NO: 4 - DNA, 35 bp, synthetic construct
  source 1..35: mol_type = other DNA
tcgtcggcagcgtcactgggtctctctggttagac

SEQ ID NO: 5 - DNA, 31 bp, synthetic construct
  source 1..31: mol_type = other DNA
tcgtcggcagcgtcagcctgggagctctctg

SEQ ID NO: 6 - DNA, 35 bp, synthetic construct
  source 1..35: mol_type = other DNA
tcgtcggcagcgtcgaacccactgcttaagcctca

SEQ ID NO: 7 - DNA, 35 bp, synthetic construct
  source 1..35: mol_type = other DNA
tcgtcggcagcgtcagcttgccttgagtgcttcaa

SEQ ID NO: 8 - DNA, 32 bp, synthetic construct
  source 1..32: mol_type = other DNA
tcgtcggcagcgtctgtgtgcccgtctgttgt

SEQ ID NO: 9 - DNA, 38 bp, synthetic construct
  source 1..38: mol_type = other DNA
tcgtcggcagcgtcctggtaactagagatccctcagac

SEQ ID NO: 10 - DNA, 38 bp, synthetic construct
  source 1..38: mol_type = other DNA
  modified_base 26: mod_base = OTHER; note = locked nucleic acid
  modified_base 29: mod_base = OTHER; note = locked nucleic acid
  modified_base 34: mod_base = OTHER; note = locked nucleic acid
tcgtcggcagcgtcagtcagtgtggaaaatctctagca

SEQ ID NO: 11 - DNA, 301 bp, synthetic construct
  source 1..301: mol_type = other DNA
cctttaagaccaatgacttacaaggcagctgtagatcttagccactttttaaaagaaaaggggggactggaagggctaattcactcccaacgaagacaagatctgctttttgcttgtactgggtctctctggttagaccagatctgagcctgggagctctctggctaactagggaacccactgcttaagcctcaataaagcttgccttgagtgcttcaagtagtgtgtgcccgtctgttgtgtgactctggtaactagagatccctcagacccttttagtcagtgtggaaaatctctagca

SEQ ID NO: 12 - DNA, 301 bp, synthetic construct; identical to SEQ ID NO: 11
  source 1..301: mol_type = other DNA

SEQ ID NO: 13 - DNA, 301 bp, synthetic construct; identical to SEQ ID NO: 11
  source 1..301: mol_type = other DNA

SEQ ID NO: 14 - DNA, 301 bp, synthetic construct; identical to SEQ ID NO: 11
  source 1..301: mol_type = other DNA

SEQ ID NO: 15 - DNA, 301 bp, synthetic construct; identical to SEQ ID NO: 11
  source 1..301: mol_type = other DNA

SEQ ID NO: 16 - DNA, 301 bp, synthetic construct; identical to SEQ ID NO: 11
  source 1..301: mol_type = other DNA

SEQ ID NO: 17 - DNA, 301 bp, synthetic construct; identical to SEQ ID NO: 11
  source 1..301: mol_type = other DNA

SEQ ID NO: 18 - DNA, 301 bp, synthetic construct; identical to SEQ ID NO: 11
  source 1..301: mol_type = other DNA

SEQ ID NO: 19 - DNA, 301 bp, synthetic construct; identical to SEQ ID NO: 11
  source 1..301: mol_type = other DNA

SEQ ID NO: 20 - DNA, 301 bp, synthetic construct; identical to SEQ ID NO: 11
  source 1..301: mol_type = other DNA

SEQ ID NO: 21 - DNA, 300 bp, synthetic construct
  source 1..300: mol_type = other DNA
tcgtcggcagcgtcgcagctgtagatcttagccactttttaaaagaaaaggggggactggaagggctaattcactcccaacgaagacaagatctgctttttgcttgtactgggtctctctggttagaccagatctgagcctgggagctctctggctaactagggaacccactgcttaagcctcaataaagcttgccttgagtgcttcaagtagtgtgtgcccgtctgttgtgtgactctggtaactagagatccctcagacccttttagtcagtgtggaaaatctctagcannnnnnnnn

SEQ ID NO: 22 - DNA, 262 bp, synthetic construct
  source 1..262: mol_type = other DNA
tcgtcggcagcgtcgggactggaagggctaattcactcccaacgaagacaagatctgctttttgcttgtactgggtctctctggttagaccagatctgagcctgggagctctctggctaactagggaacccactgcttaagcctcaataaagcttgccttgagtgcttcaagtagtgtgtgcccgtctgttgtgtgactctggtaactagagatccctcagacccttttagtcagtgtggaaaatctctagcannnnnnnnn

SEQ ID NO: 23 - DNA, 238 bp, synthetic construct
  source 1..238: mol_type = other DNA
tcgtcggcagcgtcccaacgaagacaagatctgctttttgcttgtactgggtctctctggttagaccagatctgagcctgggagctctctggctaactagggaacccactgcttaagcctcaataaagcttgccttgagtgcttcaagtagtgtgtgcccgtctgttgtgtgactctggtaactagagatccctcagacccttttagtcagtgtggaaaatctctagcannnnnnnnn

SEQ ID NO: 24 - DNA, 228 bp, synthetic construct
  source 1..228: mol_type = other DNA
tcgtcggcagcgtcactgggtctctctggttagacactgggtctctctggttagaccagatctgagcctgggagctctctggctaactagggaacccactgcttaagcctcaataaagcttgccttgagtgcttcaagtagtgtgtgcccgtctgttgtgtgactctggtaactagagatccctcagacccttttagtcagtgtggaaaatctctagcannnnnnnnn

SEQ ID NO: 25 - DNA, 195 bp, synthetic construct
  source 1..195: mol_type = other DNA
tcgtcggcagcgtcagcctgggagctctctgagcctgggagctctctggctaactagggaacccactgcttaagcctcaataaagcttgccttgagtgcttcaagtagtgtgtgcccgtctgttgtgtgactctggtaactagagatccctcagacccttttagtcagtgtggaaaatctctagcannnnnnnnn

SEQ ID NO: 26 - DNA, 151 bp, synthetic construct
  source 1..151: mol_type = other DNA
tcgtcggcagcgtcgaacccactgcttaagcctcaataaagcttgccttgagtgcttcaagtagtgtgtgcccgtctgttgtgtgactctggtaactagagatccctcagacccttttagtcagtgtggaaaatctctagcannnnnnnnn

SEQ ID NO: 27 - DNA, 126 bp, synthetic construct
  source 1..126: mol_type = other DNA
tcgtcggcagcgtcagcttgccttgagtgcttcaagtagtgtgtgcccgtctgttgtgtgactctggtaactagagatccctcagacccttttagtcagtgtggaaaatctctagcannnnnnnnn

SEQ ID NO: 28 - DNA, 101 bp, synthetic construct
  source 1..101: mol_type = other DNA
tcgtcggcagcgtctgtgtgcccgtctgttgtgtgactctggtaactagagatccctcagacccttttagtcagtgtggaaaatctctagcannnnnnnnn

SEQ ID NO: 29 - DNA, 77 bp, synthetic construct
  source 1..77: mol_type = other DNA
tcgtcggcagcgtcctggtaactagagatccctcagacccttttagtcagtgtggaaaatctctagcannnnnnnnn

SEQ ID NO: 30 - DNA, 47 bp, synthetic construct
  source 1..47: mol_type = other DNA
tcgtcggcagcgtcagtcagtgtggaaaatctctagcannnnnnnnn

SEQ ID NO: 31 - DNA, 21 bp, synthetic construct
  source 1..21: mol_type = other DNA
cccactgcttaagcctcaata

SEQ ID NO: 32 - DNA, 21 bp, synthetic construct
  source 1..21: mol_type = other DNA
gggtctgagggatctctagtt

SEQ ID NO: 33 - skipped

SEQ ID NO: 34 - DNA, 15 bp, synthetic construct
  source 1..15: mol_type = other DNA
gtgcccgtctgttgt